European Patent Application EP 4 703 470 A1, published March 4, 2026. Title: Cellulase variants. Applicant: AB Enzymes. Application EP. The sequence listing filed with the application follows.

SEQUENCE LISTING (7 sequences)

SEQ ID NO: 1 - protein, 415 aa, Achaetomium strumarium
QKPGSAKEVHPKITTYRCSNRGGCKAQTNYIVLDSLAHPIHQATSLANNCGDWGSKPNATACPDKESCAKNCIMEGIPDYSQYGVTTQGTALRLQQLLDGRLVTPRVYLLDKSEQRYEMMHLAGAEFAFEVDAAKLPCGMNSALYLSEMHPTGARSKLNPGGAYYGTGYCDAQCFVTPFINGVGNIEGHGSCCNEMDIWEANARATHLAPHPCNKPGLYLCSGDDECGDDGVCDKDGCAWNPYRVNVTDYYGASARFRVDTTRPFTVVTQFLTSTPNPPQNGKGHNKKKELTKIHRLYVQDDKVIESYTVDAPGLPKTDSLTDEFCGATGAAKYLALGGTRGIGEALERGMVLAMSIWWDEGGNMNWLDSGEAGPCDPWEGNPANITKVEPGPEVTFRNLRWGEIGSTFGDRVRL

SEQ ID NO: 2 - DNA, 1248 bp, Achaetomium strumarium
  source 1..1248: mol_type = other DNA
cagaagcctggctccgcgaaggaagtccacccgaagatcacgacctaccgctgcagcaaccgaggcggctgcaaggcccagacgaactatatcgtcctggatagcctcgcccacccaatccaccaggccacttctctggccaacaactgcggcgactggggctctaagccgaacgctacggcctgccctgataaggagagctgcgctaagaactgcatcatggagggcatcccggactactcccagtacggcgtgaccactcagggcactgccctgcgcttgcagcagctgcttgacggccgcttggtcacgccgcgtgtctacctcctggataagtccgagcagcgctacgagatgatgcacctggctggcgccgagtttgcgttcgaggtcgacgccgctaagcttccctgcggcatgaactctgctctctacctgtctgagatgcaccctacgggcgcccgcagcaagctgaacccaggcggcgcttactacggcactggctactgcgacgcccagtgcttcgtcaccccctttatcaacggcgtcggcaacatcgagggccacggcagctgctgcaacgagatggacatctgggaggccaacgctcgtgccacccacctcgcgccccacccatgcaacaagccaggcctgtacctttgctccggcgacgatgagtgcggcgatgacggcgtctgcgacaaggacggctgcgcctggaacccctatcgcgtcaacgtgacggattactatggcgcctctgctcgatttcgtgtggacactacccgtcccttcaccgtggtcacgcagttccttaccagcactccaaaccctccgcagaacggcaagggccacaacaagaagaaggagctcaccaagattcaccgactctatgtccaggacgataaggtcatcgagtcgtatactgtggacgctcccggcctgccaaagactgactcgttgactgacgagttctgcggcgctacgggcgctgccaagtaccttgctctgggcggcacgcgtggcattggcgaggctcttgagcgaggcatggtccttgctatgtcgatctggtgggacgagggcggcaacatgaactggctggattcgggcgaggccggcccctgcgatccttgggagggcaaccctgccaacattacgaaggtcgagcccggccctgaggtcacgtttcgcaacctccgctggggcgagatcggcagcacctttggcgaccgcgtgcgtctttaa

SEQ ID NO: 3 - protein, 428 aa, Melanocarpus albomyces
MTRNIALLGAASALLGLAHGQKPGETPEVHPQLTTFRCTKADGCQPRTNYIVLDSLSHPVHQVDNDYNCGDWGQKPNATACPDVESCARNCIMEGVPDYSQHGVTTSDTSLRLQQLVDGRLVTPRVYLLDETEHRYEMMHLTGQEFTFEVDATKLPCGMNSALYLSEMDPTGARSELNPGGAYYGTGYCDAQCFVTPFINGIGNIEGKGSCCNEMDIWEANSRATHVAPHTCNQTGLYMCEGAECEYDGVCDKDGCGWNPYRVNITDYYGNSDAFRVDTRRPFTVVTQFPADAEGRLESIHRLYVQDGKVIESYVVDAPGLPRTDSLNDEFCAATGAARYLDLGGTAGMGDAMTRGMVLAMSIWWDESGFMNWLDSGEAGPCLPDEGDPKNIVKVEPSPEVTYSNLRWGEIGSTFEAESDDDGDGDDC

SEQ ID NO: 4 - protein, 4 aa, synthetic construct
NRRG

SEQ ID NO: 5 - protein, 5 aa, synthetic construct
NDTTG

SEQ ID NO: 6 - protein, 14 aa, synthetic construct
STPNPPQNGKGHNK

SEQ ID NO: 7 - protein, 12 aa, synthetic construct
PNPPQNGKGHNK